European Patent Specification EP 4 053 152 B1, published June 17, 2026. Title: KERATIN BD-13, PREPARATION METHOD THEREFOR AND PHARMACEUTICAL COMPOSITION AND USE THEREOF. Applicant: Institute of Materia Medica, Chinese Academy of Medical Sciences. The sequence listing filed with the application follows.

SEQUENCE LISTING (2 sequences)

SEQ ID NO: 1 - protein, 486 aa, Bos taurus
MTCGSYRALPAFSCVSACGPRPGRCCITAAPYRGISCYRGLTGGFGSRSVCGGFRAGYCGRSFGYRSGGVGGLSPPCITTVSVNESLLTPLNLEIDPNAQCVKQEEKEQIKCLNNRFAAFIDKVRFLEQQNKLLETKLQFYQNRQCCESNLEPLFNGYIETLRREAECVEADSGRLSSELNSLQEVLEGYKKKYEEEVSLRATAENEFVALKKDVDCAYLRKSDLEANVEALIQEIDFLRRLYEEEIRVLQAHISDTSVIVKMDNSRDLNMDNIVAEIKAHYDDIASRSRAEAESWYRSKCEEIKATVIRHGETLRRTKEEINELNRTIQRLTAEVENAKCQNSKLEAAVTQAEQQGEAALNDAKCKLAGLEEALQKAKQDMACLLKEYQEVMNSKLGLDIEIATYRRLLEGEEQRLCEGVGSVNVCVSSSRGGVVCGDLCASGAAPAVTTSVCSAPCSGNVVVGTSDACGPCSRVGGSILGCKKC

SEQ ID NO: 2 - DNA, 1461 bp, Bos taurus
atgacctgcgggagctatcgtgcgctgccggcgtttagctgcgtgagcgcgtgcggcccgcgtccgggccgttgctgcattaccgcggcgccctatcgtggcataagctgctatcgtggcctgaccggcggctttggcagccgtagcgtgtgcggcggctttcgtgcgggctactgcggccgtagttttggctatcgtagcggcggcgtgggcggcctgagcccgccgtgtattaccaccgtgagcgtgaatgaaagcctgctgaccccgctgaacctggaaatagatccgaatgcgcaatgcgtgaaacaggaggagaaagagcagataaaatgtctgaacaatcgttttgcggcgttcatagataaagtccgctttctggaacagcagaacaaactgctggaaaccaaactgcagttctatcagaatcgtcagtgctgtgaaagcaacctggagccgctgttcaacggctatattgaaaccctgcgtcgtgaagcggaatgcgtggaagcggatagcggccgtttaagcagcgaactgaactcgcttcaggaagtcctggaaggctataaaaagaaatacgaggaggaagtcagccttcgtgccaccgcggaaaatgaatttgttgcactgaaaaaagatgtggactgcgcgtatctgcgtaaaagcgatttggaagcgaatgtggaagcgctgattcaggagattgattttctgcgtcgtctgtacgaagaagagattcgtgttctgcaggcgcatattagcgataccagcgtgatagtgaagatggataatagccgcgatctgaacatggacaatatcgtggcggaaatcaaggcgcattacgatgatattgcgagccgttcgcgtgcggaagcggagtcatggtatcgttcaaagtgcgaggagattaaagcgaccgtaattcgtcatggcgaaacgctgcgccgtaccaaagaagaaataaatgagctgaatcgtaccatccagcgtctgaccgcggaagtcgaaaatgcgaaatgtcagaatagcaaactggaagcggcggtgacccaggcggaacagcagggcgaggcggcgctgaatgatgcgaaatgcaaactggcgggcctggaagaagcgttgcagaaagcgaaacaggatatggcgtgcttgctgaaagaatatcaggaggtcatgaatagcaaactgggcctggatatagaaattgccacctaccgtcgcctgcttgaaggcgaggaacagcgtctgtgcgaaggcgtgggcagcgtgaatgtgtgcgtgagcagcagccgtggcggcgtggtgtgcggcgatctgtgcgcgagcggtgcggcgccggcggtgaccaccagcgtgtgcagcgcgccgtgcagcggcaatgtggtggtgggcaccagcgatgcatgcggcccgtgcagccgtgtgggcggcagcattctgggctgcaaaaaatgctaa